European Patent Specification EP 4 236 771 B1, published March 12, 2025. Title: HIGH-TRANSCONDUCTANCE ORGANIC ELECTROCHEMICAL TRANSISTOR (OECT)-BASED SENSORS AND METHODS OF USE. Applicant: The Regents of the University of California. Application PCT/US 21/56712. The sequence listing filed with the application follows.

SEQUENCE LISTING (1 sequence)

SEQ ID NO: 1 - DNA, 58 bp, Artificial Sequence
  Aptamer
gggacagggctagcagtaggattgggtgaggggatgtgctgtggaggcaaagcttccg